European Patent Specification EP 3 592 772 B1, published March 20, 2024. Title: Anti CCL24 (eotaxin2) antibodies for use in the treatment of hepatic diseases. Applicant: ChemomAb Ltd. The sequence listing filed with the application follows.

SEQUENCE LISTING (12 sequences)

SEQ ID NO: 1 - protein, 5 aa, Homo sapiens
NSGMN

SEQ ID NO: 2 - protein, 17 aa, Homo sapiens
WINTYNGEPTYTDDFKG

SEQ ID NO: 3 - protein, 11 aa, Homo sapiens
HSYGSSYAMDN

SEQ ID NO: 4 - protein, 15 aa, Homo sapiens
KASQSVDYDGDSYMN

SEQ ID NO: 5 - protein, 7 aa, Homo sapiens
VASNLKS

SEQ ID NO: 6 - protein, 9 aa, Homo sapiens
QQSNEEPWT

SEQ ID NO: 7 - protein, 120 aa, Homo sapiens
QIQLVQSGPELKKPGASVKVSCRASGYPFTNSGMNWVKQAPGKGLKWMGWINTYNGEPTYTDDFKGRFAFSLETSASTAYLQINNLRNEDTATYFCASHSYGSSYAMDNWGQGTSVTVSS

SEQ ID NO: 8 - protein, 111 aa, Homo sapiens
DIVLTQSPDSLAVSLGERATINCKASQSVDYDGDSYMNWYQQKPGQPPKLLIYVASNLKSGIPARFSGSGSGTDFTLTISSLQPEDFATYYCQQSNEEPWTFGGGTKVEIK

SEQ ID NO: 9 - DNA, 426 bp, Mus musculus
  misc_feature (11)..(11): n is a, c, g, t or u
  misc_feature (19)..(19): n is a, c, g, t or u
  misc_feature (21)..(21): n is a, c, g, t or u
  misc_feature (33)..(33): n is a, c, g, t or u
  misc_feature (39)..(40): n is a, c, g, t or u
  misc_feature (42)..(42): n is a, c, g, t or u
  misc_feature (386)..(386): n is a, c, g, t or u
  misc_feature (422)..(422): n is a, c, g, t or u
gggcagcaganccggggcngnggatagacagangggggnngncgttttggctgaggagacggtgactgaggttccttgaccccagttgtccatagcgtagctactaccgtaggaatgacttgcacagaaatatgtagccgtgtcctcatttctgaggttgttgatctgcaaataggcagtgctggcagaggtttccaaagagagggcaaaccgtcccttgaagtcatcagtatatgttggctctccattgtaggtgttgatccagcccatccactttaaaccctttcctggagcctgctttacccagttcattccagagtttgtgaagggatacccagaagccctgcaggagatcttgactgtgtctccaggcttcttcagctcangtccagactgcaccaactggatctgggccatggccngcta

SEQ ID NO: 10 - DNA, 254 bp, Mus musculus
  misc_feature (11)..(12): n is a, c, g, or t
  misc_feature (35)..(36): n is a, c, g, or t
  misc_feature (44)..(44): n is a, c, g, or t
  misc_feature (49)..(52): n is a, c, g, or t
  misc_feature (55)..(56): n is a, c, g, or t
  misc_feature (60)..(61): n is a, c, g, or t
  misc_feature (64)..(64): n is a, c, g, or t
  misc_feature (66)..(66): n is a, c, g, or t
  misc_feature (69)..(69): n is a, c, g, or t
  misc_feature (72)..(73): n is a, c, g, or t
  misc_feature (75)..(78): n is a, c, g, or t
  misc_feature (80)..(83): n is a, c, g, or t
  misc_feature (85)..(86): n is a, c, g, or t
  misc_feature (88)..(92): n is a, c, g, or t
  misc_feature (95)..(95): n is a, c, g, or t
  misc_feature (98)..(98): n is a, c, g, or t
  misc_feature (100)..(101): n is a, c, g, or t
  misc_feature (107)..(109): n is a, c, g, or t
  misc_feature (111)..(113): n is a, c, g, or t
  misc_feature (115)..(115): n is a, c, g, or t
  misc_feature (119)..(121): n is a, c, g, or t
  misc_feature (125)..(126): n is a, c, g, or t
  misc_feature (131)..(137): n is a, c, g, or t
  misc_feature (139)..(142): n is a, c, g, or t
  misc_feature (145)..(149): n is a, c, g, or t
  misc_feature (153)..(154): n is a, c, g, or t
  misc_feature (157)..(157): n is a, c, g, or t
  misc_feature (159)..(159): n is a, c, g, or t
  misc_feature (163)..(166): n is a, c, g, or t
  misc_feature (168)..(168): n is a, c, g, or t
  misc_feature (171)..(173): n is a, c, g, or t
  misc_feature (178)..(178): n is a, c, g, or t
  misc_feature (180)..(181): n is a, c, g, or t
  misc_feature (183)..(185): n is a, c, g, or t
  misc_feature (187)..(191): n is a, c, g, or t
  misc_feature (196)..(200): n is a, c, g, or t
  misc_feature (202)..(202): n is a, c, g, or t
  misc_feature (204)..(204): n is a, c, g, or t
  misc_feature (206)..(206): n is a, c, g, or t
  misc_feature (214)..(214): n is a, c, g, or t
  misc_feature (216)..(218): n is a, c, g, or t
  misc_feature (221)..(226): n is a, c, g, or t
  misc_feature (233)..(234): n is a, c, g, or t
  misc_feature (236)..(236): n is a, c, g, or t
gggccaatggnngaggacgcggatgggggtgtcgnngtgccttngtcgnnnnctnnttgnncancntcnacnncnnnnannnnanngnnnnntgnaananngatggnnntnnncnacannntggnntcctnnnnnnntnnnntgnnnnngacnncananacannnncnacnnnatgancnncnnncnnnnnttgannnnngncnantatgaacnannnaannnnnntacctgnnangccactcacaagacatca

SEQ ID NO: 11 - DNA, 360 bp, Homo sapiens
cagatccaattggtgcagtctggacctgagctgaagaagcctggagcctcagtcaaggtctcctgcagggcttctgggtatcccttcacaaactctggaatgaactgggtaaagcaggctccaggaaagggtttaaagtggatgggctggatcaacacctacaatggagagccaacatatactgatgacttcaagggacggtttgccttctctttggaaacctctgccagcactgcctatttgcagatcaacaacctcagaaatgaggacacggctacatatttctgtgcaagtcattcctacggtagtagctacgctatggacaactggggtcaaggaacctcagtcaccgtctcctca

SEQ ID NO: 12 - DNA, 333 bp, Homo sapiens
gacattgtgctgacccaatctccagactctttggctgtgtctctaggggagagggccaccatcaactgcaaggccagccaaagtgttgattatgatggtgatagttatatgaactggtaccaacagaaaccaggacagccacccaaactcctcatctatgttgcatccaatctaaaatctggcatcccagccaggtttagtggcagtgggtctgggacagacttcaccctcaccatcagcagcctgcagcctgaggattttgcaacctattactgtcagcaaagtaatgaggaaccgtggacgttcggtggaggcaccaaggtggaaatcaaa